European Patent Application EP 4 112 732 A1, published January 4, 2023. Title: NOVEL FLAVONE HYDROXYLASES, MICROORGANISM FOR SYNTHESIZING FLAVONE C-GLYCOSIDE COMPOUNDS, AND USE THEREOF. Applicant: CAS CENTER FOR EXCELLENCE IN MOLECULAR PLANT SCIENCES. The sequence listing filed with the application follows.

SEQUENCE LISTING (27 sequences)

SEQ ID NO: 1 - protein, 517 aa, Phyllostachys edulis
MAMELVALVLAAMLLLTVIMRRYGGSAGSSKHGRLPPSPMALPFIGHLHLIRPPPHRAFDRIIARHGPLIYLRLGPSTHCVVVGSADVARDFLRFEASIPERPLTAVTRQLAYGSAGFAFAPYGPHWRFMKRLCMSELLGPRTVEQLRPVRDAELAGVLRAVRAAAERGESVDMSRELIRMSNNAIMRMVASALPGDMAEAARDCAKQVAELVGAFNVEDYVAMCRGWDLQGIGRRTREVHARFDALLETMIRAKEEARRDPLPRDKSRTTKDLLDILMDVAEDEAAEVRLTRENIKAFVLDIFTAGSDTTATSVEWMLAELINHPAYLEKLRAEVDAVVGGSRLVGEPDVAQMPYLQAVLKETLRLRPPAVFAQRETIEAVHVCGYTIPPKTSVFFNIFSIGRDPACWEDPLEFRPERFMPGGASAGVDPKGQHQQLMPFGSGRRACPGMGLAMQAVPAFLAALVQCFDWAVPLPQGTPLDMEEAEGLVSARKQPLVLVPTQRLRPLPAGAAAALA

SEQ ID NO: 2 - protein, 522 aa, Phyllostachys edulis
MGDVPLPLLLGSLAVSALVWYVLFRRGGGEGAKRPPGPRGWPVLGNLPQLGAKPHHTMCAMAREYGPLFRLRFGSAEVVVAASAGVAAQFLRGLDANFSNRPPNSGAEHVAYNYQDLVFAPYGARWRALRKLCALHLFSAKALDDLRAVREGEVALLVRELARAAAGGVPAVALGQEANVTATNTLARATVGRRVFAVDGGEGAREFKEMVVELMQLAGVFNVGDFVPALRWLDPQGVVAKMKRLHRRYDDMLNGFIKERKAVVKPDGLSGGDQGKDLLSVLLARMREEQPLDGEDGKITETDIKALLLNLFTAGTDTTSSTVEWALAELIRHPDVLKQAQHELDAVAGRDRLVSESDLPRLTFLAAVIKETFRLHPSTPLSLPRVAAEECTVDGYRVPKGTTLLVNVWAIARDPASWPNPLDFNPARFLPGGTHESVDLKGSDFELIPFGAGRRVCAGLSWGLRMVTLMTATLVHAFDWALVDGMTPDKLNMEEAYGLTLQRAVPLMVQPAPRLLPSAYGM

SEQ ID NO: 3 - DNA, 27 bp, Primer
tataccatgggtgactgcgttgccccg

SEQ ID NO: 4 - DNA, 30 bp, Primer
cgggatccttacttcggcaggtcgccgctc

SEQ ID NO: 5 - DNA, 29 bp, Primer
cgggatcccttatgcgactcctgcattag

SEQ ID NO: 6 - DNA, 26 bp, Primer
gcccaagcttttatgccagcatcttc

SEQ ID NO: 7 - DNA, 31 bp, Primer
agatatacatatggttacggtggaagaatac

SEQ ID NO: 8 - DNA, 30 bp, Primer
ccgctcgagttaggtagccacactatgcag

SEQ ID NO: 9 - DNA, 30 bp, Primer
ccgctcgagctagaaataattttgtttaac

SEQ ID NO: 10 - DNA, 28 bp, Primer
gagcctaggttagttaccgattttaaag

SEQ ID NO: 11 - DNA, 38 bp, Primer
ctcccaccaggacctagcatgcgtagcgcgggtagccg

SEQ ID NO: 12 - DNA, 43 bp, Primer
tcgaattcggatccactagtttagctataaaagctcggcagcg

SEQ ID NO: 13 - DNA, 34 bp, Primer
agctcccaccaggacctagcatgggcagcgcggg

SEQ ID NO: 14 - DNA, 34 bp, Primer
tcgaattcggatccactagtttacgccagcgccg

SEQ ID NO: 15 - DNA, 46 bp, Primer
ataagaaggagatatacatatgtcctcttcttcttcttcgtcaacc

SEQ ID NO: 16 - DNA, 55 bp, Primer
ttctttaccagactcgagttaccatacatctctaagatatcttccactcgtttgc

SEQ ID NO: 17 - DNA, 36 bp, Primer
tgccgcgcggcagccatatgatgggccacctggtgc

SEQ ID NO: 18 - DNA, 43 bp, Primer
tggtgctcgagtgcggccgcctagtccaacactgcaagatccc

SEQ ID NO: 19 - protein, 16 aa, Tag
MAKKTSSKGKLPPGPS

SEQ ID NO: 20 - DNA, 40 bp, Primer
agctcccaccaggacctagcatgcgtcgtggtggcggtga

SEQ ID NO: 21 - DNA, 46 bp, Primer
gagctcgaattcggatccactagtttacataccatacgcgctcggc

SEQ ID NO: 22 - DNA, 37 bp, Primer
agctcccaccaggacctagcatgctgcgtggtggcag

SEQ ID NO: 23 - DNA, 44 bp, Primer
gagctcgaattcggatccactagtttaaacgccatacgcgctcg

SEQ ID NO: 24 - DNA, 64 bp, Primer
ggcgtaaactagtggatccctctagaaataattttgtttaactttaagaaggagatataccatg

SEQ ID NO: 25 - DNA, 40 bp, Primer
cttaagcattatgcggccttacataccatacgcgctcggc

SEQ ID NO: 26 - DNA, 64 bp, Primer
tagctaaactagtggatccctctagaaataattttgtttaactttaagaaggagatataccatg

SEQ ID NO: 27 - DNA, 38 bp, Primer
cttaagcattatgcggccttaaacgccatacgcgctcg